European Patent Specification EP 3 423 830 B1, published June 25, 2025. Title: METHODS OF DETECTING INFLAMMATORY MARKERS AND TREATING INFLAMMATORY CONDITIONS IN COMPANION ANIMALS. Applicant: Vetica Labs, Inc. The sequence listing filed with the application follows.

SEQUENCE LISTING (36 sequences)

SEQ ID NO: 1 - DNA, 21 bp, Unidentified Bacteria Species
gctttaactgtaaacaccaac

SEQ ID NO: 2 - DNA, 20 bp, Unidentified Bacteria Species
ctactgaagcagtttcagga

SEQ ID NO: 3 - DNA, 24 bp, Unidentified Bacteria Species
gctttatctgttaataccaacatc

SEQ ID NO: 4 - DNA, 23 bp, Unidentified Bacteria Species
ttactgaagcagtttcagtaccg

SEQ ID NO: 5 - DNA, 21 bp, Unidentified Bacteria Species
gcacaagtcattaataccaac

SEQ ID NO: 6 - DNA, 21 bp, Unidentified Bacteria Species
ttaacgtaacagagacagaac

SEQ ID NO: 7 - DNA, 21 bp, Unidentified Bacteria Species
gcacaagtcattaataccaac

SEQ ID NO: 8 - DNA, 18 bp, Unidentified Bacteria Species
ttaaccctgcagcagaga

SEQ ID NO: 9 - protein, 484 aa, Unidentified Bacteria Species
MALTVNTNIASVTTQVNLNKASTAQTTSMQRLSSGLRINSAKDDAAGLQIANRLTSQINGLGQAVKNANDGISIAQTAEGAMQASTDILQKMRTLALSSATGSLSPDDRKSNNDEYQALTAELNRISATTTFGGQKLLDGSYGTKAIQVGANANETINLTLDNVSAKSIGSQQLKTGNISISKDGLAAGELAVTGNGQTKTVNYGPGASAKDVAAQLNGAIGGLTATASTEVKLDASGATAAAPANFDLTVGGSTVSFVGVTDNASLADQLKSNAAKLGISVNYDESTKNLEIKSDTGENITFAPKAGAPGVKIAAKNGSGTYGAAVPLNAAAGDKSVVTGQISLDSAKGYSIADGAGANGAGSTAALYGTGVTSVSSKKTNVSDTDVTSATNAQNAVAVIDKAIGSIDSVRSGLGATQNRLTTTVDNLQNIQKNSTAARSTVQDVDFASETAELTKQQTLQQASTAILSQANQLPSSVLKLLQ

SEQ ID NO: 10 - protein, 476 aa, Unidentified Bacteria Species
MALSVNTNIASITTQGNLTKASTAQTTSMQRLSSGLRINSAKDDAAGLQISNRLTSQINGLGQAVKNANDGISIAQTAEGAMQASTDILQKMRTLALSSATGSLSADDRKSNNDEYQALTAELTRISQTTTFGGQKLLDGSYGTKAIQVGANANETINLTLDNVAANNIGSQQVKSVAITPSATGVDAGTVTVTGNGQTKDVTVTAGDSAKTIAANLNGAIGGLTATASTEVQFSVDKTAPAANFELTVGSQKVSFVGVTDTASLADQLKSNAAKLGISVNYDESNGGSLSVKSDTGENLVFGAGDAAAQAGIKVNAKDGNGEYAASGTALTAADLYVTGAISLDSAKGYSLTGGGVTKLFSAAGTAATSVKTTIADTDVTDATKAQNALAVIDKAIGSIDSVRSGLGATQNRLQTTVDNLQNIQKNSTAARSTVQDVDFASETAELTKQQTLQQASTAILSQANQLPSSVLKLLQ

SEQ ID NO: 11 - protein, 365 aa, Unidentified Bacteria Species
MAQVINTNYLSLVTQNNLNKSQGTLGSAIERLSSGLRINSAKDDAAGQAIANRFTSNVNGLTQASRNANDGISIAQTTEGALNEINNNLQRIRELTVQAKNGTNSNSDITSIQNEVKERLDEINRISEQTQFNGVKVLSGEKSEMVIQVGTNDNETIKFNLDKVDNDTLGVASDKLFDTKTEKKGVTEAGAAIDAKDIGVTGATKYEGGTVKEYKVDGKVSADKVIFNDGTKDYLVSKSDFKLKAGTADTAEFTGSKTTEFKADAGKDVKTLNVKDDALATLDKAINTIDESRSKLGAIQNRFESTINNLNNTVNNLSASRSRILDADYATEVSNMSRGQILQQAGTSVLAQANQVPQTVLSLLR

SEQ ID NO: 12 - protein, 453 aa, Unidentified Bacteria Species
MAQVINTNSLSLITQNNINKNQSALSSSIERLSSGLRINSAKDDAAGQAIANRFTSNIKGLTQAARNANDGISLAQTTEGALSEINNNLQRVRELTVQATTGTNSDSDLSSIQDEIKSRLDEIDRVSGQTQFNGVNVLAKNGTMKIQVGANDGQTIAIDLQKIDSSTLGLNGLSVSKNSLNVSEPVTQINNAANTAPLKVDLSAVATDLGVDASSLTLSNVLDKDGNATKNYVVKSGNDYFAASVDRATGKVALNKADVEYTDPANGLTTAATQAGQFVKVSADKDGNATAFVTFQGKNYAAKAASLVDTGDATTAAQGTAATTNKVTLQLSDKAAVIGTGTAANPQFPATSATAEFAGTATNDPLALLDKAIASVDKFRSSLGAVQNRLSSAVTNLNNTTTNLSEAQSRIQDADYATEVSNMSKAQIVQQAGNSVLSKANQVPQQVLSLLQG

SEQ ID NO: 13 - protein, 572 aa, Unidentified Bacteria Species
MAQVINTNSLSLITQNNINKNQSALSSSIERLSSGLRINSAKDDAAGQAIANRFTSNIKGLTQAARNANDGISVAQTTEGALSEINNNLQRVRELTVQATTGTNSQSDLDSIQDEIKSRLDEIDRVSGQTQFNGVNVPAKDGSMKIQVGANDGQTITIDLKKIDSSTLKLTGFNVNGSGSVANTAATKADLAAAAIGTPGAADSTGAIAYTVSAGLTKTTAADVLSSLADGTTITATGVKNGFAAGATSNAYKLNKDNNTFTYDTTATTAELQSYLTPKAGDTATFSVEIGGTTQDVVLSSDGKLTAKDGSKLYIDTTGNLTQNGGNNGVGTLAEATLSGLALNNNNGAAAVKSTITTADNTSIVLNGSSNGTEGTIAVTGAVISSAALQSASKTTGFTVGTADTAGYISVGTDGSVQAYDVATSGNKDSYTNTDGTLTTDNTTKLYLQKDGSVTNGSGKAVYVEADGDFTTDAATKAATTTDPLAALDDAISQIDKFRSSLGAIQNRLDSAVTNLNNTTTNLSEAQSRIQDADYATEVSNMSKAQIIQQAGNSVLAKANQVPQQVLSLLQG

SEQ ID NO: 14 - DNA, 20 bp, Unidentified Bacteria Species
ctgaagtttacaacaaagac

SEQ ID NO: 15 - DNA, 21 bp, Unidentified Bacteria Species
ttagaactggtaaaccagacc

SEQ ID NO: 16 - protein, 355 aa, Unidentified Bacteria Species
AEVYNKDGNKLDLYGKVDGLHYFSDNKSEDGDQTYVRLGFKGETQVTDQLTGYGQWEYQIQGNTSEDNKENSWTRVAFAGLKFQDVGSFDYGRNYGVVYDVTSWTDVLPEFGGDTYGSDNFMQQRGNGFATYRNTDFFGLVDGLNFAVQYQGKNGSVSGEGMTNNGRGALRQNGDGVGGSITYDYEGFGIGAAVSSSKRTDDQNGSYTSNGVVRNYIGTGDRAETYTGGLKYDANNIYLAAQYTQTYNATRVGSLGWANKAQNFEAVAQYQFDFGLRPSLAYLQSKGKNLGVINGRNYDDEDILKYVDVGATYYFNKNMSTYVDYKINLLDDNQFTRDAGINTDNIVALGLVYQF

SEQ ID NO: 17 - protein, 346 aa, Unidentified Bacteria Species
AEVYNKDGNKLDLYGKVDGLHYFSDNKDVDGDQTYMRLGFKGETQVTDQLTGYGQWEYQIQGNSAENENNSWTRVAFAGLKFQDVGSFDYGRNYGVVYDVTSWTDVLPEFGGDTYGSDNFMQQRGNGFATYRNTDFFGLVDGLNFAVQYQGKNGSVSGEGMTNNGRGALRQNGDGVGGSITYDYEGFGIGGAISSSKRTDDQNSPLYIGNGDRAETYTGGLKYDANNIYLAAQYTQTYNATRVGSLGWANKAQNFEAVAQYQFDFGLRPSVAYLQSKGKNLGVINGRNYDDEDILKYVDVGATYYFNKNMSTYVDYKINLLDDNQFTRDAGINTDNIVALGLVYQF

SEQ ID NO: 18 - protein, 343 aa, Unidentified Bacteria Species
AEVYNKDGNKLDLYGKVDGLHYFSDNDSKDGDKTYMRLGFKGETQVTDQLTGYGQWEYQIQGNEPESDNSSWTRVAFAGLKFQDVGSFDYGRNYGVVYDVTSWTDVLPEFGGDTYDSDNFMQQRGNGFATYRNTDFFGLVDGLDFAVQYQGKNGSAHGEGMTTNGRDDVFEQNGDGVGGSITYNYEGFGIGAAVSSSKRTWDQNNTGLIGTGDRAETYTGGLKYDANNIYLAAQYTQTYNATRVGSLGWANKAQNFEAVAQYQFDFGLRPSLAYLQSKGKNLGRGYDDEDILKYVDVGATYYFNKNMSTYVDYKINLLDDNRFTRDAGINTDDIVALGLVYQF

SEQ ID NO: 19 - protein, 243 aa, Artificial Sequence
  Hetero-chimeric S100A8/S100A9
MGSSHHHHHHGLTELESAINSLIEVYHKYSLVKGNYHALYRDDLKKLLETECPQYMKKKDADTWFQELDVNSDGAINFEEFLILVIKVGVASHKDIHKEGGGGSGGGGSGGGGSADQMSQLECSIETIINIFHQYSVRLEHPDKLNQKEMKQLVKKELPNFLKKQKKNDNAINKIMEDLDTNGDKELNFEEFSILVARLTVASHEEMHKNAPEGEGHSHGPGFGEGSQGHCHSHGGHGHGHSH

SEQ ID NO: 20 - protein, 102 aa, Artificial Sequence
  S100A12
MGSSHHHHHHGTKLEDHLEGIVDVFHRYSARVGHPDTLSKGEMKQLIIRELPNTLKNTKDQATVDKLFQDLDADKDGQVNFNEFISLVSVVLDTSHKNTHKE

SEQ ID NO: 21 - protein, 99 aa, Artificial Sequence
  S100A8
MGSSHHHHHHGLTELESAINSLIEVYHKYSLVKGNYHALYRDDLKKLLETECPQYMKKKDADTWFQELDVNSDGAINFEEFLILVIKVGVASHKDIHKE

SEQ ID NO: 22 - protein, 140 aa, Artificial Sequence
  S100A9
  misc_feature (130)..(130): Xaa can be any naturally occurring amino acid
MGSSHHHHHHGADQMSQLECSIETIINIFHQYSVRLEHPDKLNQKEMKQLVKKELPNFLKKQKKNDNAINKIMEDLDTNGDKELNFEEFSILVARLTVASHEEMHKNAPEGEGHSHGPGFGEGSQGFFIXHGGHGHGHSH

SEQ ID NO: 23 - DNA, 21 bp, Unidentified Bacteria Species
gtgtctgcctctcgacctcgg

SEQ ID NO: 24 - DNA, 27 bp, Unidentified Bacteria Species
cagagaattgaaggatttcaaatcagc

SEQ ID NO: 25 - DNA, 27 bp, Unidentified Bacteria Species
ttatgtgaaatgacgtttgggtctttg

SEQ ID NO: 26 - DNA, 21 bp, Unidentified Bacteria Species
gaattggatgccaagatctcc

SEQ ID NO: 27 - DNA, 27 bp, Unidentified Bacteria Species
ttacagtgtgtgcagctccacagtcag

SEQ ID NO: 28 - DNA, 24 bp, Unidentified Bacteria Species
ttagtgatccgcgcctctctcttg

SEQ ID NO: 29 - protein, 909 aa, Unidentified Bacteria Species
WLVVGAPTARWLANASVVNPGAIYRCRIGGNPGLTCEQLQLGSPSGEPCGKTCLEERDNQWLGVTLSRQPGENGSIVTCGHRWKNIFYIKNENKLPMGVCYGMPSDLRTELSKRIAPCYQDYVRKFGENFASCQAGISSFYTEDLIVMGAPGSSYWTGSLFVYNITTNKYKAFLDRQNQVKFGSYLGYSVGAGHFRSPHTTEVVGGAPQHEQIGKAYIFSIEAKELSILHEMKGKKLGSYFGASVCAVDLNADGFSDLLVGAPMQSTIREEGRVFVYINSGSGAVMNEMETELIGSDKYAARFGESIVNLGDIDNDGFEDVAVGAPQEDDLRGAVYIYNGRADGISTAFSQRIEGFQISKSLSMFGQSISGQIDADNNGYVDVAVGAFRSDSAVLLRTRPVVIVEVSLNHPESVNRTNFDCVENGLPSVCMDLTLCFSYKGKEVPGYIVLLYNMSLDVNRKIDSPSRFYFSSNGTSDVITGSMKVSSKVPNCRTHQAFMRKDVRDILTPIQIEAAYRLGQHVIRKRSTEEFPPLQPILQQKKERDIIEKTINFARFCAHENCSADLQVSARIGFLKPHENKTYVAVGSMKTVMLNVSLFNAGDDAYETALHIRLPSGLYFIKILDLEEKQINCEVTDSSGSVKLDCSIGYIYMDRLSRMDISFLLDVSSLSQAEEDLSLTVHATCANEREMDNLNKVTLAIPLKYEVMLSVHGFVNPTSFIYGPKEENEPDTCMAEKMNFTFHVINTGHSMAPNVSVEIMVPNSFAPQTDKLFNILDVQPAGECHFKTYQRKCALEQEKGAMKILKDIFTFLSKTDKKLLFCMKADPYCLTILCHLGKMESGKEASVHIQLEGRPYLSEMDETSALKFEVRVTAFPEPNPKVIELNKDENVAHVLLEGLHHQRPKRHFT

SEQ ID NO: 30 - protein, 1015 aa, Unidentified Bacteria Species
VSASRPRPGSTPPPPPWQVYPVAEAWEGGASSSGSGEQGPRAGGCGAPAGSSPKVLVAKSGARGLSSSWWGRRGDAQARGFGAGSWELEGDLAHVCAHLHGCPLGLWLVVGAPTARWLANASVVNPGAIYRCRIGGNPGLTCEQLQLGSPSGEPCGKTCLEERDNQWLGVTLSRQPGENGSIVTCGHRWKNIFYIKNENKLPMGVCYGMPSDLRTELSKRIAPCYQDYVRKFGENFASCQAGISSFYTEDLIVMGAPGSSYWTGSLFVYNITTNKYKAFLDRQNQVKFGSYLGYSVGAGHFRSPHTTEVVGGAPQHEQIGKAYIFSIEAKELSILHEMKGKKLGSYFGASVCAVDLNADGFSDLLVGAPMQSTIREEGRVFVYINSGSGAVMNEMETELIGSDKYAARFGESIVNLGDIDNDGFEDVAVGAPQEDDLRGAVYIYNGRADGISTAFSQRIEGFQISKSLSMFGQSISGQIDADNNGYVDVAVGAFRSDSAVLLRTRPVVIVEVSLNHPESVNRTNFDCVENGLPSVCMDLTLCFSYKGKEVPGYIVLLYNMSLDVNRKIDSPSRFYFSSNGTSDVITGSMKVSSKVPNCRTHQAFMRKDVRDILTPIQIEAAYRLGQHVIRKRSTEEFPPLQPILQQKKERDIIEKTINFARFCAHENCSADLQVSARIGFLKPHENKTYVAVGSMKTVMLNVSLFNAGDDAYETALHIRLPSGLYFIKILDLEEKQINCEVTDSSGSVKLDCSIGYIYMDRLSRMDISFLLDVSSLSQAEEDLSLTVHATCANEREMDNLNKVTLAIPLKYEVMLSVHGFVNPTSFIYGPKEENEPDTCMAEKMNFTFHVINTGHSMAPNVSVEIMVPNSFAPQTDKLFNILDVQPAGECHFKTYQRKCALEQEKGAMKILKDIFTFLSKTDKKLLFCMKADPYCLTILCHLGKMESGKEASVHIQLEGRPYLSEMDETSALKFEVRVTAFPEPNPKVIELNKDENVAHVLLEGLHHQRPKRHFT

SEQ ID NO: 31 - protein, 440 aa, Unidentified Bacteria Species
ELDAKISSAEKATEWRDPDLSLLGSCQPAPSCRECILSHPSCAWCKQLFWGLGIRDQDASPFGSWGGPSPWPAHRCRPALWCLFCDPPPPPPASAPRLSPGPSRRCTLDPLLCRRLHRAPCALCPAPCTLHPALRLGTPCATSTWPARPLAQPSPCPLPGFGSFVDKTVLPFVSTVPAKLRHPCPTRLERCQPPFSFRHVLSLTGDATAFEREVGRQSVSGNLDSPEGGFDAILQAALCQEKIGWRNVSRLLVFTSDDTFHTAGDGKLGGIFMPSDGHCHLDSNGLYSRSPEFDYPSVGQVAQALSTANIQPIFAVTSATLPVYQELSKLIPKSAVGELSEDSSNVVQLIMDAYNSLSSTVTLEHSALPPGVHISYESLCGDPEKREAEAGDRGQCSHVPINHTVNFLVTLQATRCLPEPHLLRLRALGFSEELTVELHL

SEQ ID NO: 32 - protein, 691 aa, Unidentified Bacteria Species
ELDAKISSAEKATEWRDPDLSLLGSCQPAPSCRECILSHPSCAWCKQLFWGLGIRDQDASPFGSWGGPSPWPAHRCRPALWCLFCDPPPPPPASAPRLSPGPSRRCTLDPLLCRRLHRAPCALCPAPCTLHPALRLGTPCATSTWPARPLAQPSPCPLPGFGSFVDKTVLPFVSTVPAKLRHPCPTRLERCQPPFSFRHVLSLTGDATAFEREVGRQSVSGNLDSPEGGFDAILQAALCQEKIGWRNVSRLLVFTSDDTFHTAGDGKLGGIFMPSDGHCHLDSNGLYSRSPEFDYPSVGQVAQALSTANIQPIFAVTSATLPVYQELSKLIPKSAVGELSEDSSNVVQLIMDAYNSLSSTVTLEHSALPPGVHISYESLCGDPEKREAEAGDRGQCSHVPINHTVNFLVTLQATRCLPEPHLLRLRALGFSEELTVELHTLCDCNCSDTQPQAPHCSDGQGLLQCGVCSCAPGRLGRLCECSEAELSSPDLESGCRAPNGTGPLCSGKGRCQCGRCSCSGQSSGPLCECDDASCERHEGILCGGFGHCQCGRCHCHANRTGSACECSMDTDSCLGPEGEVCSGHGDCKCNRCQCRDGYFGALCEQCSGCKTSCERHRDCAECGAFGTGPLATNCSVACAHYNVTLALVPVLDDGWCKERTLDNQLLFFLVEEEAGGMVVLTVRPQERGADH

SEQ ID NO: 33 - protein, 119 aa, Artificial Sequence
  TAG
MGSSHHHHHHGSGLVPRGSASMSDSEVNQEAKPEVKPEVKPETHINLKVSDGSSEIFFKIKKTTPLRRLMEAFAKRQGKEMDSLRFLYDGIRIQADQTPEDLDMEDNDIIEAHREQIGG

SEQ ID NO: 34 - protein, 602 aa, Artificial Sequence
  Flagellin
MGSSHHHHHHGSGLVPRGSASMSDSEVNQEAKPEVKPEVKPETHINLKVSDGSSEIFFKIKKTTPLRRLMEAFAKRQGKEMDSLRFLYDGIRIQADQTPEDLDMEDNDIIEAHREQIGGALTVNTNIASVTTQVNLNKASTAQTTSMQRLSSGLRINSAKDDAAGLQIANRLTSQINGLGQAVKNANDGISIAQTAEGAMQASTDILQKMRTLALSSATGSLSPDDRKSNNDEYQALTAELNRISATTTFGGQKLLDGSYGTKAIQVGANANETINLTLDNVSAKSIGSQQLKTGNISISKDGLAAGELAVTGNGQTKTVNYGPGASAKDVAAQLNGAIGGLTATASTEVKLDASGATAAAPANFDLTVGGSTVSFVGVTDNASLADQLKSNAAKLGISVNYDESTKNLEIKSDTGENITFAPKAGAPGVKIAAKNGSGTYGAAVPLNAAAGDKSVVTGQISLDSAKGYSIADGAGANGAGSTAALYGTGVTSVSSKKTNVSDTDVTSATNAQNAVAVIDKAIGSIDSVRSGLGATQNRLTTTVDNLQNIQKNSTAARSTVQDVDFASETAELTKQQTLQQASTAILSQANQLPSSVLKLLQ

SEQ ID NO: 35 - protein, 474 aa, Artificial Sequence
  OMPC
MGSSHHHHHHGSGLVPRGSASMSDSEVNQEAKPEVKPEVKPETHINLKVSDGSSEIFFKIKKTTPLRRLMEAFAKRQGKEMDSLRFLYDGIRIQADQTPEDLDMEDNDIIEAHREQIGGAEVYNKDGNKLDLYGKVDGLHYFSDNKSEDGDQTYVRLGFKGETQVTDQLTGYGQWEYQIQGNTSEDNKENSWTRVAFAGLKFQDVGSFDYGRNYGVVYDVTSWTDVLPEFGGDTYGSDNFMQQRGNGFATYRNTDFFGLVDGLNFAVQYQGKNGSVSGEGMTNNGRGALRQNGDGVGGSITYDYEGFGIGAAVSSSKRTDDQNGSYTSNGVVRNYIGTGDRAETYTGGLKYDANNIYLAAQYTQTYNATRVGSLGWANKAQNFEAVAQYQFDFGLRPSLAYLQSKGKNLGVINGRNYDDEDILKYVDVGATYYFNKNMSTYVDYKINLLDDNQFTRDAGINTDNIVALGLVYQF

SEQ ID NO: 36 - protein, 11 aa, Artificial Sequence
  Poly-His tag
MGSSHHHHHHG